European Patent Application EP 4 289 955 A1, published December 13, 2023. Title: Protein with transport activity of fucose-containing carbohydrates and Method for producing fucose-containing carbohydrates. Applicant: KYOWA HAKKO BIO CO., LTD. The sequence listing filed with the application follows.

SEQUENCE LISTING (48 sequences)

SEQ ID NO: 1 - DNA, 1191 bp, Escherichia coli
atgacaacaaacactgtttcccgcaaagtggcgtggctacgggtcgttacgctggcagtcgccgccttcatcttcaacaccaccgaatttgtccctgttggcctgctctctgacattgcgcaaagttttcacatgcaaaccgctcaggtcggcatcatgttgaccatttacgcatgggtagtagcgctaatgtcattgccttttatgttaatgaccagtcaggttgaacggcgcaaattactgatctgcctgtttgtggtgtttattgccagccacgtactgtcgtttttgtcgtggagctttaccgttctggtgatcagtcgcattggtgtggcttttgcacatgcgattttctggtcgattacggcgtctctggcgatccgtatggctccggccgggaagcgagcacaggcattgagtttaattgccaccggtacagcactggcgatggtcttaggtttacctctcgggcgcattgtgggccagtatttcggttggcgaatgaccttcttcgcgattggtattggggcgcttatcacccttttgtgcctgattaagttacttcccttactgcccagtgagcattccggttcactgaaaagcctcccgctattgttccgccgcccggcattgatgagcatttatttgttaactgtggtggttgtcaccgcccattacacggcatacagctatatcgagccttttgtacaaaacattgcgggattcagcgccaactttgccacggcattactgttattactcggtggtgcgggcattattggcagcgtgattttcggtaaactgggtaatcagtatgcgtctgcgttggtgagtacggcgattgcgctgttgctggtgtgcctggcattgctgttacctgcggcgaacagtgaaatacacctcggggtgctgagtattttctgggggatcgcgatgatgatcatcgggcttggtatgcaggttaaagtgctggcgctggcaccagatgctaccgacgtcgcgatggcgctattctccggcatatttaatattggaatcggggcgggtgcgttggtaggtaatcaggtgagtttgcactggtcaatgtcgatgattggttatgtgggcgcggtgcctgcttttgccgcgttaatttggtcaatcattatatttcgccgctggccagtgacactcgaagaacagacgcaatag

SEQ ID NO: 2 - protein, 396 aa, Escherichia coli
MTTNTVSRKVAWLRVVTLAVAAFIFNTTEFVPVGLLSDIAQSFHMQTAQVGIMLTIYAWVVALMSLPFMLMTSQVERRKLLICLFVVFIASHVLSFLSWSFTVLVISRIGVAFAHAIFWSITASLAIRMAPAGKRAQALSLIATGTALAMVLGLPLGRIVGQYFGWRMTFFAIGIGALITLLCLIKLLPLLPSEHSGSLKSLPLLFRRPALMSIYLLTVVVVTAHYTAYSYIEPFVQNIAGFSANFATALLLLLGGAGIIGSVIFGKLGNQYASALVSTAIALLLVCLALLLPAANSEIHLGVLSIFWGIAMMIIGLGMQVKVLALAPDATDVAMALFSGIFNIGIGAGALVGNQVSLHWSMSMIGYVGAVPAFAALIWSIIIFRRWPVTLEEQTQ

SEQ ID NO: 3 - DNA, 1233 bp, Escherichia coli
atgcaaaataaattagcttccggtgccaggcttggacgtcaggcgttacttttccctctctgtctggtgctttacgaattttcaacctatatcggcaacgatatgattcaacccggtatgttggccgtggtggaacaatatcaggcgggcattgattgggttcctacttcgatgaccgcgtatctggcgggcgggatgtttttacaatggctgctggggccgctgtcggatcgtattggtcgccgtccggtgatgctggcgggagtggtgtggtttatcgtcacctgtctggcaatattgctggcgcaaaacattgaacaattcaccctgttgcgcttcttgcagggcataagcctctgtttcattggcgctgtgggatacgccgcaattcaggaatccttcgaagaggcggtttgtatcaagatcaccgcgctgatggcgaacgtggcgctgattgctccgctacttggtccgctggtgggcgcggcgtggatccatgtgctgccctgggaggggatgtttgttttgtttgccgcattggcagcgatctcctttttcggtctgcaacgagccatgcctgaaaccgccacgcgtataggcgagaaactgtcactgaaagaactcggtcgtgactataagctggtgctgaagaacggccgctttgtggcgggggcgctggcgctgggattcgttagtctgccgttgctggcgtggatcgcccagtcgccgattatcatcattaccggcgagcagttgagcagctatgaatatggcttgctgcaagtgcctattttcggggcgttaattgcgggtaacttgctgttagcgcgtctgacctcgcgccgcaccgtacgttcgctgattattatgggcggctggccgattatgattggtctattggtcgctgctgcggcaacggttatctcatcgcacgcgtatttatggatgactgccgggttaagtatttatgctttcggtattggtctggcgaatgcgggactggtgcgattaaccctgtttgccagcgatatgagtaaaggtacggtttctgccgcgatgggaatgctgcaaatgctgatctttaccgttggtattgaaatcagcaaacatgcctggctgaacgggggcaacggactgtttaatctcttcaaccttgtcaacggaattttgtggctgtcgctgatggttatctttttaaaagataaacagatgggaaattctcacgaagggtaa

SEQ ID NO: 4 - protein, 410 aa, Escherichia coli
MQNKLASGARLGRQALLFPLCLVLYEFSTYIGNDMIQPGMLAVVEQYQAGIDWVPTSMTAYLAGGMFLQWLLGPLSDRIGRRPVMLAGVVWFIVTCLAILLAQNIEQFTLLRFLQGISLCFIGAVGYAAIQESFEEAVCIKITALMANVALIAPLLGPLVGAAWIHVLPWEGMFVLFAALAAISFFGLQRAMPETATRIGEKLSLKELGRDYKLVLKNGRFVAGALALGFVSLPLLAWIAQSPIIIITGEQLSSYEYGLLQVPIFGALIAGNLLLARLTSRRTVRSLIIMGGWPIMIGLLVAAAATVISSHAYLWMTAGLSIYAFGIGLANAGLVRLTLFASDMSKGTVSAAMGMLQMLIFTVGIEISKHAWLNGGNGLFNLFNLVNGILWLSLMVIFLKDKQMGNSHEG

SEQ ID NO: 5 - DNA, 954 bp, Artificial Sequence
  Description of the artificial sequence: base sequence of Chimera-type FucT
atgaaattgaaagtgaaatttgtagatttttgggatggctttgatgaacattataatactttcgttaatgttctatctgagaaatatgaaatcgaaatttgtgatcatcctgattacttaatatattcgacttttggatataagaacttaaagtacgaaaattgtgttaagatattttatacgggtgaaaatataactccagactttaatctttgtgattatgcgattggctttgatataatggaattcggagatcgctatatgcgcctaccattatatgccttatatggtattgaagagttgcgtaaacctaaagtctttaattcacaggaagctctgaatcgtaagttctgcagcatcgtggttagcaataataaatgggcggacccgattcgtgagacctttttcaaactgctgagcagctacaaaaaggtggacagcggtggccgtgcgtggaacaacatcggtggcccggttgacaacaagctggatttcatcagccagtacaaattcaacattgcgtttgagaacagccgtgtgctgggttacaccaccgaaaagattatggagccgatgcaagtgaacagcattccggtttactggggtaacagattggttgagttggattttaatcctaattcttttattaatgctgcagattacccatctttagaagctttggtagaatatatcgttgagttggacacaaatgatgataaatatctgtcaattttgtcaagaccttggcttaacaaaagtaattatttggattggcaagaaaggctttttagcttctttgagaatgttttcaataaaccattgaatgaacagaaatatttatcaccttatgggtacggtaagctatatagaagaagattaatggaaatgtatattgcgaaaagaaaattgaaaaaatggaaaatggtttgtaacccttgtcgttggtttagatga

SEQ ID NO: 6 - protein, 317 aa, Artificial Sequence
  Description of the artificial sequence: amino acid sequence of Chimera-type FucT
MKLKVKFVDFWDGFDEHYNTFVNVLSEKYEIEICDHPDYLIYSTFGYKNLKYENCVKIFYTGENITPDFNLCDYAIGFDIMEFGDRYMRLPLYALYGIEELRKPKVFNSQEALNRKFCSIVVSNNKWADPIRETFFKLLSSYKKVDSGGRAWNNIGGPVDNKLDFISQYKFNIAFENSRVLGYTTEKIMEPMQVNSIPVYWGNRLVELDFNPNSFINAADYPSLEALVEYIVELDTNDDKYLSILSRPWLNKSNYLDWQERLFSFFENVFNKPLNEQKYLSPYGYGKLYRRRLMEMYIAKRKLKKWKMVCNPCRWFR

SEQ ID NO: 7 - DNA, 264 bp, Artificial Sequence
  Description of the artificial sequence: partial base sequence of codon-optimized BfFucT
cgtaagttctgcagcatcgtggttagcaataataaatgggcggacccgattcgtgagacctttttcaaactgctgagcagctacaaaaaggtggacagcggtggccgtgcgtggaacaacatcggtggcccggttgacaacaagctggatttcatcagccagtacaaattcaacattgcgtttgagaacagccgtgtgctgggttacaccaccgaaaagattatggagccgatgcaagtgaacagcattccggtttactggggt

SEQ ID NO: 8 - DNA, 20 bp, Artificial Sequence
  Description of the artificial sequence: base sequence of primer for amplification of cat
accaggcgtttaagggcacc

SEQ ID NO: 9 - DNA, 45 bp, Artificial Sequence
  Description of the artificial sequence: base sequence of primer for amplification of cat
gactacgggcctaaagtcgacagaataaataaatcctggtgtccc

SEQ ID NO: 10 - DNA, 28 bp, Artificial Sequence
  Description of the artificial sequence: base sequence of primer for amplification of sacB
gtcgactttaggcccgtagtctgcaaat

SEQ ID NO: 11 - DNA, 21 bp, Artificial Sequence
  Description of the artificial sequence: base sequence of primer for amplification of sacB
tacggttagccatttgcctgc

SEQ ID NO: 12 - DNA, 42 bp, Artificial Sequence
  Description of the artificial sequence: base sequence of primer for amplification of lacZ Upstream 1
ggtgcccttaaacgcctggtagctgtttcctgtgtgaaattg

SEQ ID NO: 13 - DNA, 18 bp, Artificial Sequence
  Description of the artificial sequence: base sequence of primer for amplification of lacZ Upstream 1
ccagtctggccctgcacg

SEQ ID NO: 14 - DNA, 43 bp, Artificial Sequence
  Description of the artificial sequence: base sequence of primer for amplification of lacY Downstream 1
gcaggcaaatggctaaccgtacgaccaacatatcataacggag

SEQ ID NO: 15 - DNA, 20 bp, Artificial Sequence
  Description of the artificial sequence: base sequence of primer for amplification of lacY Downstream 1
gtttccgctctgtttgctgc

SEQ ID NO: 16 - DNA, 42 bp, Artificial Sequence
  Description of the artificial sequence: base sequence of primer for amplification of  lacZ Upstream 2
ccgttatgatatgttggtcgagctgtttcctgtgtgaaattg

SEQ ID NO: 17 - DNA, 22 bp, Artificial Sequence
  Description of the artificial sequence: base sequence of amplification primer for amplification of lacY Downstream 2
cgaccaacatatcataacggag

SEQ ID NO: 18 - DNA, 41 bp, Artificial Sequence
  Description of the artificial sequence: base sequence of primer for amplification of wcaJ Upstream 1
ggtgcccttaaacgcctggtcgttgttcctgttattagccc

SEQ ID NO: 19 - DNA, 20 bp, Artificial Sequence
  Description of the artificial sequence: base sequence of primer for amplification of wcaJ Upstream 1
acgcggtcgctatcagcaaa

SEQ ID NO: 20 - DNA, 44 bp, Artificial Sequence
  Description of the artificial sequence: base sequence of primer for amplification of wcaM Downstream 1
gcaggcaaatggctaaccgtaatttgcgaccattcctggaaaaa

SEQ ID NO: 21 - DNA, 23 bp, Artificial Sequence
  Description of the artificial sequence: base sequence of primer for amplification of wcaM Downstream 1
acttcacaaacgcctgcatatag

SEQ ID NO: 22 - DNA, 41 bp, Artificial Sequence
  Description of the artificial sequence: base sequence of primer for amplification of wcaJ Upstream 2
ttccaggaatggtcgcaaatcgttgttcctgttattagccc

SEQ ID NO: 23 - DNA, 23 bp, Artificial Sequence
  Description of the artificial sequence: base sequence of primer for amplification of wcaM Downstream 2
atttgcgaccattcctggaaaaa

SEQ ID NO: 24 - DNA, 26 bp, Artificial Sequence
  Description of the artificial sequence: base sequence of primer for amplification of rcsA
atgtcaacgattattatggatttatg

SEQ ID NO: 25 - DNA, 42 bp, Artificial Sequence
  Description of the artificial sequence: base sequence of primer for amplification of rcsA
cattctagacctccttaattagcgcatgttgacaaaaatacc

SEQ ID NO: 26 - DNA, 38 bp, Artificial Sequence
  Description of the artificial sequence: base sequence of primer for amplification of cBrFucT Upstream
aggaggtctagaatgaaattgaaagtgaaatttgtaga

SEQ ID NO: 27 - DNA, 35 bp, Artificial Sequence
  Description of the artificial sequence: base sequence of primer for amplification of cBrFucT Downstream
ggatttcctctcgagtcatctaaaccaacgacaag

SEQ ID NO: 28 - DNA, 22 bp, Artificial Sequence
  Description of the artificial sequence: base sequence of primer for amplification of cBrFucT Upstream
attcagagcttcctgtgaatta

SEQ ID NO: 29 - DNA, 41 bp, Artificial Sequence
  Description of the artificial sequence: base sequence of primer for amplification of cBrFucT Middlestream
attcacaggaagctctgaatcgtaagttctgcagcatcgtg

SEQ ID NO: 30 - DNA, 20 bp, Artificial Sequence
  Description of the artificial sequence: base sequence of primer for amplification of cBrFucT Middlestream
accccagtaaaccggaatgc

SEQ ID NO: 31 - DNA, 40 bp, Artificial Sequence
  Description of the artificial sequence: base sequence of primer for amplification of cBrFucT Downstream
gcattccggtttactggggtaacagattggttgagttgga

SEQ ID NO: 32 - DNA, 45 bp, Artificial Sequence
  Description of the artificial sequence: base sequence of primer for amplification of lacY
ctcgagaggaaatccattatgtactatttaaaaaacacaaacttt

SEQ ID NO: 33 - DNA, 23 bp, Artificial Sequence
  Description of the artificial sequence: base sequence of primer for amplification of lacY
ttaagcgacttcattcacctgac

SEQ ID NO: 34 - DNA, 41 bp, Artificial Sequence
  Description of the artificial sequence: base sequence of primer for amplification of rcsA-cBrFucT-lacY
gaggagaaattaaccatgtcaacgattattatggatttatg

SEQ ID NO: 35 - DNA, 38 bp, Artificial Sequence
  Description of the artificial sequence: base sequence of primer for amplification of rcsA-cBrFucT-lacY
agggcatcggtcgacttaagcgacttcattcacctgac

SEQ ID NO: 36 - DNA, 21 bp, Artificial Sequence
  Description of the artificial sequence: base sequence of primer for amplification of pPE167
gtcgaccgatgcccttgagag

SEQ ID NO: 37 - DNA, 25 bp, Artificial Sequence
  Description of the artificial sequence: base sequence of primer for amplification of pPE167
ggttaatttctcctctttaatatcg

SEQ ID NO: 38 - DNA, 36 bp, Artificial Sequence
  Description of the artificial sequence: base sequence of primer for amplification of pSTV29
ggaaggagtaacactatgaccatgattacgccaagc

SEQ ID NO: 39 - DNA, 34 bp, Artificial Sequence
  Description of the artificial sequence: base sequence of primer for amplification of pSTV29
accacaaaagcggttaacgccatgagcggcctca

SEQ ID NO: 40 - DNA, 20 bp, Artificial Sequence
  Description of the artificial sequence: base sequence of primer for amplification of PuspA
aaccgcttttgtggtgacca

SEQ ID NO: 41 - DNA, 22 bp, Artificial Sequence
  Description of the artificial sequence: base sequence of primer for amplification of PuspA
agtgttactccttccataaagt

SEQ ID NO: 42 - DNA, 20 bp, Artificial Sequence
  Description of the artificial sequence: base sequence of primer for amplification of pSTV-PuspA
gaattcactggccgtcgttt

SEQ ID NO: 43 - DNA, 38 bp, Artificial Sequence
  Description of the artificial sequence: base sequence of primer for amplification of ydeA
ggaaggagtaacactatgacaacaaacactgtttcccg

SEQ ID NO: 44 - DNA, 36 bp, Artificial Sequence
  Description of the artificial sequence: base sequence of primer for amplification of ydeA
acggccagtgaattcctattgcgtctgttcttcgag

SEQ ID NO: 45 - DNA, 18 bp, Artificial Sequence
  Description of the artificial sequence: base sequence of primer for amplification of pMW118
accctggcgttacccaac

SEQ ID NO: 46 - DNA, 20 bp, Artificial Sequence
  Description of the artificial sequence: base sequence of primer for amplification of pMW118
agctgtttcctgtgtgaaat

SEQ ID NO: 47 - DNA, 39 bp, Artificial Sequence
  Description of the artificial sequence: base sequence of primer for amplification of mdfA
acacaggaaacagctatgcaaaataaattagcttccggt

SEQ ID NO: 48 - DNA, 36 bp, Artificial Sequence
  Description of the artificial sequence: base sequence of primer for amplification of mdfA
gggtaacgccagggtttacccttcgtgagaatttcc